European Patent Application EP 4 349 962 A1, published April 10, 2024. Title: BACTERIAL STRAIN HSCY 2073, ISOLATION AND SCREENING THEREOF, AND APPLICATION THEREOF IN IMPROVEMENT ON FLAVOR QUALITY OF VINEGAR. Applicant: Jiangsu Hengshun Vinegar-industry Co., Ltd. The sequence listing filed with the application follows.

SEQUENCE LISTING (1 sequence)

SEQ ID NO: 1 - DNA, 1540 bp, Lactobacillus sp.HSCY 2073(Lactobacillus sp. HSCY 2073)
agagtttgatcctggctcaggatgaacgctggcggtgtgcctaatacatgcaagtcgcgcgcactcccgtagatgattttgatgctctgcatcaaatgattctacattcgagtgagcggcggatgggtgagtaacacgtgggtaacctgcccttgagtctgggatagcatctggaaacggataataataccggataacaactgaaaccacatggtttcagtttgaaaggcgcgtttgcgtcgctcttggagggacccgcggtccattagttagttggtaagataaaggcctaccaagacgatgatggatagccgaactgagaggttgatcggccacattggaactgagacacggtccagactcctacgggaggcagcagtagggaatctttcacaatgggcgaaagcctgatgaagcaacaccgcgtgaatgaagaagggtttcggctcgtaaaattctgttgctagagaagaacgtaccaagtaggaaatggcttggtagtgacggtatctggttagaaagtcacggctaactacgtgccagcagccgcggtaatacgtaggtggcaagcgttatccggatttattgggcgtaaagcgagcgcaggcggttgtttaagtccgatgtgaaagccttcggcttaaccgaagaagtgcattggaaactgagcgacttgagtacagaagaggacagtagaacaccatgtgtagcggtgaaatgcgtagatatatggtagaataccagtggcgaaagcggctgtctggtctgtcactgacgctgaggctcgaaagcatgggtagcaaacaggattagataccctggtagtccatgctgtaaacgttgagtgctaggtgttagaggatttccgtcctttagtgccgaagttaacacattaagcactccgcctggggagtacgaccgcaaggttgaaactcaaaggaattgacggggacccgcacaagtggtggagcatgtggtttaattcgatgctacgcgaagaaccttaccaggccttgacatacttctgttaggctaagagattagctgttcccttcggggacagatctacaggtggtgcatggtcgtcgtcagctcgtgtcgtgagatgttgggtcaagtcccgcaacgagcacaacccttgtgactagttgccagcattcagttgggcactctagtcagactgccggtgataaaccggaggaaggtgaggatgacgtctgatcatcatgccccttatggcctgggctacacacgtgctacaatggacagtacaatgggttgcgaaaccgcgaggtcaagcttatcccataaagctgttctcagttcggactgcagtctgcaactcgactgcacgaagctggaatcactagtaatcgtggatcagcatgccacggtgaatacgttcccgggtcttgtacataccgcccgtcacaccatgagagtccgtaacacccaaagatagtgcggcaacctcttttgaggagccagctatctaaggtgggacgaatgattagggtgaagtcgtaacaacgtagccgta